European Patent Application EP 4 582 107 A1, published July 9, 2025. Title: An agent for preventing aggravation of uremia in a feline suffering from a severe renal failure. Applicant: 宮崎　徹. The sequence listing filed with the application follows.

SEQUENCE LISTING (6 sequences)

SEQ ID NO: 1 - protein, 355 aa, Felis catus
MALLFSLILAIYTGPGILGSFSRVRLVGGDHRCEGRVELQQDDEWVTVCDDYWNMDSVAVLCRELGCGAARKTMSGTVYGPVTPKDQKVFIHLFRCNGIEESLSQCEREDAIGCSHVEDAGAVCEPIYTGPGILGPESVRLADGPGRCQGRVEVKFRGEWSSVCQAGWSFAAAKVVCRQLGCGRATLTRRGCNKATQGQGAIWQRKASCSGQEVSLQDCLSEVWEHNCTHNEDVWVECEDPFALKLVGGRSHCEGRLEVLHKGEWGSVCDDGWGQDADRVVCRQLGCGQPLSPPVKVRRRFGPGVGRIWLDDVKCSGKEPSLEQCLHRSWGYHNCNHREDVAVVCEEQQSGLPDA

SEQ ID NO: 2 - DNA, 1068 bp, Felis catus
  source 1..1068: mol_type = other DNA
  misc_feature 1..1068: note = cDNA encoding Cat AIM
atggcgctactcttctccctaatcctcgccatttacactggacctggcattttagggtctttttccagagtgcggctagtgggaggcgaccaccgctgtgaaggtcgtgtggagttgcagcaggatgacgagtgggtcaccgtgtgtgatgactactggaacatggactctgtggccgtgctgtgccgggagctgggctgtggggcggccaggaagaccatgagtggcaccgtgtatggaccagtgacaccaaaggaccaaaaagtcttcatccacctgttcagatgcaatgggatcgaagaaagcctgtctcagtgcgagagggaagatgcaatcggatgctcccatgttgaggatgcgggagccgtgtgcgagcccatttacactggacctggcattttagggccggagagtgtgaggctggccgatggccccgggcgctgccagggccgagtggaggtgaagttccgaggggagtggagctctgtgtgccaagcaggctggagctttgcagccgccaaggtggtgtgccggcagctggggtgtggacgggccaccctgacccggagaggctgcaacaaagcgacccagggccaaggggccatctggcagagaaaggcgtcatgctcaggacaagaagtgagccttcaagattgcctttctgaagtttgggaacacaactgtacccacaatgaggacgtgtgggtcgaatgtgaagatccctttgccttgaagctggtaggaggacgcagccactgtgaggggaggctggaggtgctgcacaagggcgagtggggctctgtctgcgacgacggctggggacaagacgcagaccgggtggtgtgcaggcagctgggctgcgggcagcccctgtctccgcctgtcaaagtccggagaaggttcggccccggggtcggccgcatctggctggacgacgtcaagtgctcggggaaggagccgtccctggagcagtgcctgcacaggtcctggggctaccacaactgtaaccacagagaggatgtggctgtggtctgtgaagaacagcagtctggcctacctgatgcttga

SEQ ID NO: 3 - protein, 352 aa, Mus musculus
MAPLFNLMLAILSIFVGSCFSESPTKVQLVGGAHRCEGRVEVEHNGQWGTVCDDGWDRRDVAVVCRELNCGAVIQTPRGASYQPPASEQRVLIQGVDCNGTEDTLAQCELNYYVFDCSHEEDAGAQCENPDSDLLFIPEDVRLVDGPGHCQGRVEVLHQSQWSTVCKAGWNLQVSKVVCRQLGCGRALLTYGSCNKNTQGKGPIWMGKMSCSGQEANLRSCLLSRLENNCTHGEDTWMECEDPFELKLVGGDTPCSGRLEVLHKGSWGSVCDDNWGEKEDQVVCKQLGCGKSLHPSPKTRKIYGPGAGRIWLDDVNCSGKEQSLEFCRHRLWGYHDCTHKEDVEVICTDFDV

SEQ ID NO: 4 - DNA, 1059 bp, Mus musculus
  source 1..1059: mol_type = other DNA
  misc_feature 1..1059: note = cDNA encoding mouse AIM
atggctccattgttcaacttgatgctggccatcttgagcatttttgttggatcgtgtttttcagagtctccaaccaaagtgcagctagtgggaggtgcccaccgctgtgaagggcgagtggaggtggaacacaatggccagtgggggactgtgtgtgatgatggctgggaccggcgtgatgtggctgtggtgtgccgagagctcaattgtggagcagtcatccaaaccccgcgtggcgcatcatatcagccaccagcatcagagcaaagagttcttattcaaggggttgactgcaacggaacggaagacacgttggctcaatgtgagctaaattacgatgtttttgactgctcacatgaagaagatgctggggcacagtgtgagaacccagacagtgacctcctcttcattccagaggatgtgcgtctagtagatggcccggggcactgccagggtcgagtggaggtgctccaccagtcccagtggagcactgtgtgtaaagcaggctggaacttacaggtctcaaaggtggtgtgcaggcagctcgggtgtgggcgggcattactgacctacggaagctgcaacaagaatactcagggcaaaggacccatctggatgggcaagatgtcgtgttctggacaagaagcaaaccttcggtcttgccttttgagtcgtttggagaacaactgtacccatggcgaggacacatggatggaatgtgaagatccttttgagctgaagctggtgggaggagacaccccctgctctgggaggttggaggtgctgcacaagggttcctggggctccgtctgtgatgacaactggggagaaaaggaggaccaagtggtctgcaagcaactgggttgtgggaagtccctccatccatcccccaaaacccggaaaatctatgggcctggggcaggccgcatctggctggatgacgtcaactgctcagggaaggaacagtctctggagttctgccggcacaggttgtgggggtaccacgactgtacccacaaggaagatgtggaggtgatctgcacagactttgatgtgtga

SEQ ID NO: 5 - protein, 347 aa, Homo sapiens
MALLFSLILAICTRPGFLASPSGVRLVGGLHRCEGRVEVEQKGQWGTVCDDGWDIKDVAVLCRELGCGAASGTPSGILYEPPAEKEQKVLIQSVSCTGTEDTLAQCEQEEVYDCSHDEDAGASCENPESSFSPVPEGVRLADGPGHCKGRVEVKHQNQWYTVCQTGWSLRAAKVVCRQLGCGRAVLTQKRCNKHAYGRKPIWLSQMSCSGREATLQDCPSGPWGKNTCNHDEDTWVECEDPFDLRLVGGDNLCSGRLEVLHKGVWGSVCDDNWGEKEDQVVCKQLGCGKSLSPSFRDRKCYGPGVGRIWLDNVRCSGEEQSLEQCQHRFWGFHDCTHQEDVAVICSG

SEQ ID NO: 6 - DNA, 1044 bp, Homo sapiens
  source 1..1044: mol_type = other DNA
  misc_feature 1..1044: note = cDNA encoding human AIM
atggctctgctattctccttgatccttgccatttgcaccagacctggattcctagcgtctccatctggagtgcggctggtggggggcctccaccgctgtgaagggcgggtggaggtggaacagaaaggccagtggggcaccgtgtgtgatgacggctgggacattaaggacgtggctgtgttgtgccgggagctgggctgtggagctgccagcggaacccctagtggtattttgtatgagccaccagcagaaaaagagcaaaaggtcctcatccaatcagtcagttgcacaggaacagaagatacattggctcagtgtgagcaagaagaagtttatgattgttcacatgatgaagatgctggggcatcgtgtgagaacccagagagctctttctccccagtcccagagggtgtcaggctggctgacggccctgggcattgcaagggacgcgtggaagtgaagcaccagaaccagtggtataccgtgtgccagacaggctggagcctccgggccgcaaaggtggtgtgccggcagctgggatgtgggagggctgtactgactcaaaaacgctgcaacaagcatgcctatggccgaaaacccatctggctgagccagatgtcatgctcaggacgagaagcaacccttcaggattgcccttctgggccttgggggaagaacacctgcaaccatgatgaagacacgtgggtcgaatgtgaagatccctttgacttgagactagtaggaggagacaacctctgctctgggcgactggaggtgctgcacaagggcgtatggggctctgtctgtgatgacaactggggagaaaaggaggaccaggtggtatgcaagcaactgggctgtgggaagtccctctctccctccttcagagaccggaaatgctatggccctggggttggccgcatctggctggataatgttcgttgctcaggggaggagcagtccctggagcagtgccagcacagattttgggggtttcacgactgcacccaccaggaagatgtggctgtcatctgctcaggatag